European Patent Specification EP 3 862 431 B1, published June 26, 2024. Title: Method for producing hairpin single-stranded RNA molecules. Applicant: Toray Industries, Inc. Bonac Corporation. The sequence listing filed with the application follows.

SEQUENCE LISTING (6 sequences)

SEQ ID NO: 1 - RNA, 51 nt, Artificial
  synthetic
  modified_base (24)..(25): nucleotides 24 and 25 are connected via a linker
  modified_base (50)..(51): nucleotides 50 and 51 are connected via a linker
agcagaguacacacagcauauaccgguauaugcuguguguacucugcuucg

SEQ ID NO: 2 - RNA, 24 nt, Artificial
  synthetic
  modified_base (24): nucleotide 24 is connected to a linker
agcagaguacacacagcauauacc

SEQ ID NO: 3 - RNA, 27 nt, Artificial
  synthetic
  modified_base (1): nucleotide 1 is connected to a linker
  modified_base (26)..(27): nucleotides 26 and 27 are connected via a linker
gguauaugcuguguguacucugcuucg

SEQ ID NO: 4 - RNA, 51 nt, Artificial
  synthetic
  modified_base (22)..(23): nucleotides 22 and 23 are connected via a linker
  modified_base (48)..(49): nucleotides 48 and 49 are connected via a linker
caugagaaguaugacaacagccggcuguugucauacuucucaugguucgaa

SEQ ID NO: 5 - RNA, 22 nt, Artificial
  synthetic
  modified_base (22): nucleotide 22 is connected to a linker
caugagaaguaugacaacagcc

SEQ ID NO: 6 - RNA, 29 nt, Artificial
  synthetic
  modified_base (1): nucleotide 1 is connected to a linker
  modified_base (26)..(27): nucleotides 26 and 27 are connected via a linker
ggcuguugucauacuucucaugguucgaa